European Patent Application EP 3 613 426 A9, published May 24, 2023. Title: CELL PENETRATING PEPTIDES AND METHODS OF MAKING AND USING THEREOF. Applicant: OHIO STATE INNOVATION FOUNDATION OHIO STATE INNOVATION FOUNDATION. Application EP15796259.8. The sequence listing filed with the application follows.

SEQUENCE LISTING (246 sequences)

SEQ ID NO: 1 - protein, 6 aa, Artificial Sequence
  Synthetic Construct
  MISC_FEATURE (2)..(2): L-napthylalanine
FXRRRQ

SEQ ID NO: 2 - protein, 6 aa, Artificial Sequence
  Synthetic Construct
  MISC_FEATURE (2)..(2): L-napthylalanine
FXRRRC

SEQ ID NO: 3 - protein, 6 aa, Artificial Sequence
  Synthetic Construct
  MISC_FEATURE (2)..(2): L-napthylalanine
  MISC_FEATURE (6)..(6): selenocysteine
FXRRRX

SEQ ID NO: 4 - protein, 6 aa, Artificial Sequence
  Synthetic Construct
  MISC_FEATURE (4)..(4): L-napthylalanine
RRRXFQ

SEQ ID NO: 5 - protein, 6 aa, Artificial Sequence
  Synthetic Construct
  MISC_FEATURE (5)..(5): L-napthylalanine
RRRRXF

SEQ ID NO: 6 - protein, 6 aa, Artificial Sequence
  Synthetic Construct
  MISC_FEATURE (2)..(2): L-napthylalanine
FXRRRR

SEQ ID NO: 7 - protein, 7 aa, Artificial Sequence
  Synthetic Construct
  MISC_FEATURE (2)..(2): D-napthylalanine
FXRRRRQ

SEQ ID NO: 8 - protein, 7 aa, Artificial Sequence
  Synthetic Construct
  MISC_FEATURE (2)..(2): D-napthylalanine
FXRRRRQ

SEQ ID NO: 9 - protein, 7 aa, Artificial Sequence
  Synthetic Construct
  MISC_FEATURE (2)..(2): L-napthylalanine
FXRRRRQ

SEQ ID NO: 10 - protein, 7 aa, Artificial Sequence
  Synthetic Construct
  MISC_FEATURE (2)..(2): L-napthylalanine
FXRRRRQ

SEQ ID NO: 11 - protein, 7 aa, Artificial Sequence
  Synthetic Construct
  MISC_FEATURE (5)..(5): L-napthylalanine
RRFRXRQ

SEQ ID NO: 12 - protein, 7 aa, Artificial Sequence
  Synthetic Construct
  MISC_FEATURE (6)..(6): L-napthylalanine
FRRRRXQ

SEQ ID NO: 13 - protein, 7 aa, Artificial Sequence
  Synthetic Construct
  MISC_FEATURE (5)..(5): L-napthylalanine
RRFRXRQ

SEQ ID NO: 14 - protein, 7 aa, Artificial Sequence
  Synthetic Construct
  MISC_FEATURE (3)..(3): L-napthylalanine
RRXFRRQ

SEQ ID NO: 15 - protein, 8 aa, Artificial Sequence
  Synthetic Construct
CRRRRFWQ

SEQ ID NO: 16 - protein, 8 aa, Artificial Sequence
  Synthetic Construct
  MISC_FEATURE (3)..(3): L-napthylalanine
FFXRRRRQ

SEQ ID NO: 17 - protein, 8 aa, Artificial Sequence
  Synthetic Construct
  MISC_FEATURE (3)..(3): L-napthylalanine
FFXRRRRQ

SEQ ID NO: 18 - protein, 8 aa, Artificial Sequence
  Synthetic Construct
  MISC_FEATURE (6)..(6): L-napthylalanine
RFRFRXRQ

SEQ ID NO: 19 - protein, 8 aa, Artificial Sequence
  Synthetic Construct
  MISC_FEATURE (1)..(1): selenocysteine
XRRRRFWQ

SEQ ID NO: 20 - protein, 8 aa, Artificial Sequence
  Synthetic Construct
CRRRRFWQ

SEQ ID NO: 21 - protein, 8 aa, Artificial Sequence
  Synthetic Construct
  MISC_FEATURE (2)..(2): L-napthylalanine
FXRRRRQK

SEQ ID NO: 22 - protein, 8 aa, Artificial Sequence
  Synthetic Construct
  MISC_FEATURE (2)..(2): L-napthylalanine
FXRRRRQC

SEQ ID NO: 23 - protein, 8 aa, Artificial Sequence
  Synthetic Construct
  MISC_FEATURE (2)..(2): L-napthylalanine
FXRRRRRQ

SEQ ID NO: 24 - protein, 8 aa, Artificial Sequence
  Synthetic Construct
  MISC_FEATURE (2)..(2): L-napthylalanine
FXRRRRRQ

SEQ ID NO: 25 - protein, 9 aa, Artificial Sequence
  Synthetic Construct
  MISC_FEATURE (5)..(5): L-napthylalanine
  MISC_FEATURE (8)..(8): L-norleucine
RRRRXFDXC

SEQ ID NO: 26 - protein, 5 aa, Artificial Sequence
  Synthetic Construct
  MISC_FEATURE (2)..(2): L-napthylalanine
FXRRR

SEQ ID NO: 27 - protein, 5 aa, Artificial Sequence
  Synthetic Construct
FWRRR

SEQ ID NO: 28 - protein, 5 aa, Artificial Sequence
  Synthetic Construct
  MISC_FEATURE (4)..(4): L-napthylalanine
RRRXF

SEQ ID NO: 29 - protein, 5 aa, Artificial Sequence
  Synthetic Construct
RRRWF

SEQ ID NO: 30 - protein, 5 aa, Artificial Sequence
  Synthetic Construct
RRRRR

SEQ ID NO: 31 - protein, 5 aa, Artificial Sequence
  Synthetic Construct
AAAAA

SEQ ID NO: 32 - protein, 4 aa, Artificial Sequence
  Synthetic Construct
FFFF

SEQ ID NO: 33 - protein, 5 aa, Artificial Sequence
  Synthetic Construct
  MISC_FEATURE (3)..(3): phosphocoumaryl amino propionic acid
DEXLI

SEQ ID NO: 34 - protein, 7 aa, Artificial Sequence
  Synthetic Construct
AAAAAAA

SEQ ID NO: 35 - protein, 5 aa, Artificial Sequence
  Synthetic Construct
RARAR

SEQ ID NO: 36 - protein, 5 aa, Artificial Sequence
  Synthetic Construct
DADAD

SEQ ID NO: 37 - protein, 4 aa, Artificial Sequence
  Synthetic Construct
  MISC_FEATURE (2)..(2): norleucine
  MISC_FEATURE (3)..(3): selenocysteine
DXXD

SEQ ID NO: 38 - protein, 4 aa, Artificial Sequence
  Synthetic Construct
  MISC_FEATURE (1)..(1): 2-aminobutyric acid
XTRV

SEQ ID NO: 39 - protein, 6 aa, Artificial Sequence
  Synthetic Construct
  MISC_FEATURE (2)..(2): L-homoproline
  MISC_FEATURE (4)..(4): L-4-(phosphonodifluoromethyl)phenylalanine
PXGXYR

SEQ ID NO: 40 - protein, 6 aa, Artificial Sequence
  Synthetic Construct
  MISC_FEATURE (2)..(2): L-homoproline
  MISC_FEATURE (4)..(4): L-4-(phosphonodifluoromethyl)phenylalanine
  MISC_FEATURE (5)..(5): L-4-(phosphonodifluoromethyl)phenylalanine
SXIXXR

SEQ ID NO: 41 - protein, 6 aa, Artificial Sequence
  Synthetic Construct
  MISC_FEATURE (4)..(4): L-4-(phosphonodifluoromethyl)phenylalanine
IHIXIR

SEQ ID NO: 42 - protein, 6 aa, Artificial Sequence
  Synthetic Construct
  MISC_FEATURE (4)..(4): L-4-(phosphonodifluoromethyl)phenylalanine
  MISC_FEATURE (5)..(5): L-homoproline
AAIXXR

SEQ ID NO: 43 - protein, 6 aa, Artificial Sequence
  Synthetic Construct
  MISC_FEATURE (1)..(1): L-4-fluorophenylalanine
  MISC_FEATURE (3)..(3): L-homoproline
  MISC_FEATURE (4)..(4): L-4-(phosphonodifluoromethyl)phenylalanine
XSXXVR

SEQ ID NO: 44 - protein, 6 aa, Artificial Sequence
  Synthetic Construct
  MISC_FEATURE (1)..(1): L-homoproline
  MISC_FEATURE (4)..(4): L-4-(phosphonodifluoromethyl)phenylalanine
XNPXAR

SEQ ID NO: 45 - protein, 6 aa, Artificial Sequence
  Synthetic Construct
  MISC_FEATURE (2)..(2): L-phenylglycine
  MISC_FEATURE (4)..(4): L-4-(phosphonodifluoromethyl)phenylalanine
TXAXGR

SEQ ID NO: 46 - protein, 6 aa, Artificial Sequence
  Synthetic Construct
  MISC_FEATURE (4)..(4): L-4-(phosphonodifluoromethyl)phenylalanine
AHIXAR

SEQ ID NO: 47 - protein, 6 aa, Artificial Sequence
  Synthetic Construct
  MISC_FEATURE (4)..(4): L-4-(phosphonodifluoromethyl)phenylalanine
GNGXPR

SEQ ID NO: 48 - protein, 6 aa, Artificial Sequence
  Synthetic Construct
  MISC_FEATURE (3)..(3): L-homoproline
  MISC_FEATURE (4)..(4): L-4-(phosphonodifluoromethyl)phenylalanine
FQXXIR

SEQ ID NO: 49 - protein, 6 aa, Artificial Sequence
  Synthetic Construct
  MISC_FEATURE (4)..(4): L-4-(phosphonodifluoromethyl)phenylalanine
SPGXHR

SEQ ID NO: 50 - protein, 6 aa, Artificial Sequence
  Synthetic Construct
  MISC_FEATURE (1)..(1): L-homoproline
  MISC_FEATURE (4)..(4): L-4-(phosphonodifluoromethyl)phenylalanine
XYIXHR

SEQ ID NO: 51 - protein, 6 aa, Artificial Sequence
  Synthetic Construct
  MISC_FEATURE (4)..(4): L-4-(phosphonodifluoromethyl)phenylalanine
SVPXHR

SEQ ID NO: 52 - protein, 6 aa, Artificial Sequence
  Synthetic Construct
  MISC_FEATURE (4)..(4): L-4-(phosphonodifluoromethyl)phenylalanine
AIPXNR

SEQ ID NO: 53 - protein, 6 aa, Artificial Sequence
  Synthetic Construct
  MISC_FEATURE (1)..(1): L-4-fluorophenylalanine
  MISC_FEATURE (4)..(4): L-4-(phosphonodifluoromethyl)phenylalanine
XSIXQF

SEQ ID NO: 54 - protein, 6 aa, Artificial Sequence
  Synthetic Construct
  MISC_FEATURE (3)..(3): L-phenylglycine
  MISC_FEATURE (4)..(4): L-4-(phosphonodifluoromethyl)phenylalanine
AAXXFR

SEQ ID NO: 55 - protein, 6 aa, Artificial Sequence
  Synthetic Construct
  MISC_FEATURE (3)..(3): L-phenylglycine
  MISC_FEATURE (4)..(4): L-4-(phosphonodifluoromethyl)phenylalanine
  MISC_FEATURE (5)..(5): L-phenylglycine
NTXXXR

SEQ ID NO: 56 - protein, 6 aa, Artificial Sequence
  Synthetic Construct
  MISC_FEATURE (3)..(3): L-phenylglycine
  MISC_FEATURE (4)..(4): L-4-(phosphonodifluoromethyl)phenylalanine
  MISC_FEATURE (5)..(5): L-norleucine
IPXXXR

SEQ ID NO: 57 - protein, 6 aa, Artificial Sequence
  Synthetic Construct
  MISC_FEATURE (2)..(2): L-homoproline
  MISC_FEATURE (3)..(3): L-4-fluorophenylalanine
  MISC_FEATURE (4)..(4): L-4-(phosphonodifluoromethyl)phenylalanine
  MISC_FEATURE (5)..(5): L-homoproline
QXXXXR

SEQ ID NO: 58 - protein, 6 aa, Artificial Sequence
  Synthetic Construct
  MISC_FEATURE (3)..(3): L-4-fluorophenylalanine
  MISC_FEATURE (4)..(4): L-4-(phosphonodifluoromethyl)phenylalanine
NAXXGR

SEQ ID NO: 59 - protein, 6 aa, Artificial Sequence
  Synthetic Construct
  MISC_FEATURE (4)..(4): L-4-(phosphonodifluoromethyl)phenylalanine
NTYXAR

SEQ ID NO: 60 - protein, 6 aa, Artificial Sequence
  Synthetic Construct
  MISC_FEATURE (3)..(3): L-phenylglycine
  MISC_FEATURE (4)..(4): L-4-(phosphonodifluoromethyl)phenylalanine
EAXXVR

SEQ ID NO: 61 - protein, 6 aa, Artificial Sequence
  Synthetic Construct
  MISC_FEATURE (3)..(3): L-phenylglycine
  MISC_FEATURE (4)..(4): L-4-(phosphonodifluoromethyl)phenylalanine
IVXXAR

SEQ ID NO: 62 - protein, 6 aa, Artificial Sequence
  Synthetic Construct
  MISC_FEATURE (3)..(3): L-phenylglycine
  MISC_FEATURE (4)..(4): L-4-(phosphonodifluoromethyl)phenylalanine
YTXXAR

SEQ ID NO: 63 - protein, 6 aa, Artificial Sequence
  Synthetic Construct
  MISC_FEATURE (2)..(2): L-homoproline
  MISC_FEATURE (3)..(3): L-phenylglycine
  MISC_FEATURE (4)..(4): L-4-(phosphonodifluoromethyl)phenylalanine
NXXXIR

SEQ ID NO: 64 - protein, 6 aa, Artificial Sequence
  Synthetic Construct
  MISC_FEATURE (1)..(1): L-homoproline
  MISC_FEATURE (4)..(4): L-4-(phosphonodifluoromethyl)phenylalanine
XNWXHR

SEQ ID NO: 65 - protein, 6 aa, Artificial Sequence
  Synthetic Construct
  MISC_FEATURE (2)..(2): L-homoproline
  MISC_FEATURE (4)..(4): L-4-(phosphonodifluoromethyl)phenylalanine
YXVXIR

SEQ ID NO: 66 - protein, 6 aa, Artificial Sequence
  Synthetic Construct
  MISC_FEATURE (4)..(4): X4 = L-4-(phosphonodifluoromethyl)phenylalanine
  MISC_FEATURE (4)..(4): L-4-(phosphonodifluoromethyl)phenylalanine
NSAXGR

SEQ ID NO: 67 - protein, 6 aa, Artificial Sequence
  Synthetic Construct
  MISC_FEATURE (4)..(4): L-4-(phosphonodifluoromethyl)phenylalanine
TNVXAR

SEQ ID NO: 68 - protein, 6 aa, Artificial Sequence
  Synthetic Construct
  MISC_FEATURE (4)..(4): L-4-(phosphonodifluoromethyl)phenylalanine
NTVXTR

SEQ ID NO: 69 - protein, 6 aa, Artificial Sequence
  Synthetic Construct
  MISC_FEATURE (4)..(4): L-4-(phosphonodifluoromethyl)phenylalanine
SITXYR

SEQ ID NO: 70 - protein, 6 aa, Artificial Sequence
  Synthetic Construct
  MISC_FEATURE (2)..(2): L-4-fluorophenylalanine
  MISC_FEATURE (4)..(4): L-4-(phosphonodifluoromethyl)phenylalanine
NXNXLR

SEQ ID NO: 71 - protein, 6 aa, Artificial Sequence
  Synthetic Construct
  MISC_FEATURE (4)..(4): L-4-(phosphonodifluoromethyl)phenylalanine
  MISC_FEATURE (5)..(5): L-norleucine
YNNXXR

SEQ ID NO: 72 - protein, 6 aa, Artificial Sequence
  Synthetic Construct
  MISC_FEATURE (4)..(4): L-4-(phosphonodifluoromethyl)phenylalanine
NYNXGR

SEQ ID NO: 73 - protein, 6 aa, Artificial Sequence
  Synthetic Construct
  MISC_FEATURE (4)..(4): L-4-(phosphonodifluoromethyl)phenylalanine
AWNXAR

SEQ ID NO: 74 - protein, 6 aa, Artificial Sequence
  Synthetic Construct
  MISC_FEATURE (4)..(4): L-4-(phosphonodifluoromethyl)phenylalanine
VTHXYR

SEQ ID NO: 75 - protein, 6 aa, Artificial Sequence
  Synthetic Construct
  MISC_FEATURE (2)..(2): L-phenylglycine
  MISC_FEATURE (4)..(4): L-4-(phosphonodifluoromethyl)phenylalanine
  MISC_FEATURE (5)..(5): L-homoproline
PXHXXR

SEQ ID NO: 76 - protein, 6 aa, Artificial Sequence
  Synthetic Construct
  MISC_FEATURE (2)..(2): L-phenylglycine
  MISC_FEATURE (4)..(4): L-4-(phosphonodifluoromethyl)phenylalanine
NXHXGR

SEQ ID NO: 77 - protein, 6 aa, Artificial Sequence
  Synthetic Construct
  MISC_FEATURE (4)..(4): L-4-(phosphonodifluoromethyl)phenylalanine
PAHXGR

SEQ ID NO: 78 - protein, 6 aa, Artificial Sequence
  Synthetic Construct
  MISC_FEATURE (4)..(4): L-4-(phosphonodifluoromethyl)phenylalanine
AYHXIR

SEQ ID NO: 79 - protein, 6 aa, Artificial Sequence
  Synthetic Construct
  MISC_FEATURE (2)..(2): L-homoproline
  MISC_FEATURE (4)..(4): L-4-(phosphonodifluoromethyl)phenylalanine
NXEXYR

SEQ ID NO: 80 - protein, 6 aa, Artificial Sequence
  Synthetic Construct
  MISC_FEATURE (4)..(4): L-4-(phosphonodifluoromethyl)phenylalanine
VSSXTR

SEQ ID NO: 81 - protein, 8 aa, Artificial Sequence
  Synthetic Construct
  MISC_FEATURE (2)..(2): sarcosine
  MISC_FEATURE (3)..(3): D-phosphothreonine
  MISC_FEATURE (4)..(4): L-pipecolic acid
  MISC_FEATURE (5)..(5): L-beta-naphthylalanine
AXXXXYNK

SEQ ID NO: 82 - protein, 9 aa, Artificial Sequence
  Synthetic Construct
  MISC_FEATURE (1)..(1): trimesic acid
  MISC_FEATURE (3)..(3): sarcosine
  MISC_FEATURE (4)..(4): D-phosphothreonine
  MISC_FEATURE (5)..(5): L-pipecolic acid
  MISC_FEATURE (6)..(6): L-beta-naphthylalanine
  MISC_FEATURE (9)..(9): L-2,3-diaminopropionic acid
XAXXXXRAX

SEQ ID NO: 83 - protein, 10 aa, Artificial Sequence
  Synthetic Construct
  MISC_FEATURE (1)..(1): trimesic acid
  MISC_FEATURE (3)..(3): sarcosine
  MISC_FEATURE (4)..(4): D-phosphothreonine
  MISC_FEATURE (5)..(5): L-pipecolic acid
  MISC_FEATURE (6)..(6): L-beta-naphthylalanine
  MISC_FEATURE (10)..(10): L-2,3-diaminopropionic acid
XAXXXXRAAX

SEQ ID NO: 84 - protein, 10 aa, Artificial Sequence
  Synthetic Construct
  MISC_FEATURE (1)..(1): trimesic acid
  MISC_FEATURE (3)..(3): sarcosine
  MISC_FEATURE (5)..(5): L-pipecolic acid
  MISC_FEATURE (6)..(6): L-beta-naphthylalanine
  MISC_FEATURE (10)..(10): L-2,3-diaminopropionic acid
XAXTXXRAAX

SEQ ID NO: 85 - protein, 10 aa, Artificial Sequence
  Synthetic Construct
  MISC_FEATURE (1)..(1): trimesic acid
  MISC_FEATURE (3)..(3): sarcosine
  MISC_FEATURE (6)..(6): L-beta-naphthylalanine
  MISC_FEATURE (10)..(10): L-2,3-diaminopropionic acid
XAXTAXRAAX

SEQ ID NO: 86 - protein, 9 aa, Artificial Sequence
  Synthetic Construct
  MISC_FEATURE (2)..(2): L-2-naphthylalanine
  MISC_FEATURE (9)..(9): rhodamine B
FXRRRRQKX

SEQ ID NO: 87 - protein, 9 aa, Artificial Sequence
  Synthetic Construct
  MISC_FEATURE (2)..(2): L-2-naphthylalanine
  MISC_FEATURE (9)..(9): dexamethasone
FXRRRRQKX

SEQ ID NO: 88 - protein, 16 aa, Artificial Sequence
  Synthetic Construct
  MISC_FEATURE (2)..(2): dexamethasone
KXGRKKRRQRRRPPQY

SEQ ID NO: 89 - protein, 12 aa, Artificial Sequence
  Synthetic Construct
  MISC_FEATURE (2)..(2): L-2-naphthylalanine
FXRRRRQKFITC

SEQ ID NO: 90 - protein, 14 aa, Artificial Sequence
  Synthetic Construct
  MISC_FEATURE (2)..(2): L-2-naphthylalanine
  MISC_FEATURE (14)..(14): rhodamine B
FXRRRRQRRRRRKX

SEQ ID NO: 91 - protein, 14 aa, Artificial Sequence
  Synthetic Construct
  MISC_FEATURE (2)..(2): L-2-naphthylalanine
  MISC_FEATURE (14)..(14): rhodamine B
FXRRRRQAAAAAKX

SEQ ID NO: 92 - protein, 13 aa, Artificial Sequence
  Synthetic Construct
  MISC_FEATURE (2)..(2): L-2-naphthylalanine
  MISC_FEATURE (13)..(13): rhodamine B
FXRRRRQFFFFKX

SEQ ID NO: 93 - protein, 13 aa, Artificial Sequence
  Synthetic Construct
  MISC_FEATURE (2)..(2): L-2-naphthylalanine
  MISC_FEATURE (8)..(8): 8-amino-3,6-dioxaoctanoic acid
  MISC_FEATURE (11)..(11): phosphocoumaryl amino propionic acid
FXRRRRQXDEXLI

SEQ ID NO: 94 - protein, 15 aa, Artificial Sequence
  Synthetic Construct
  MISC_FEATURE (10)..(10): 8-amino-3,6-dioxaoctanoic acid
  MISC_FEATURE (13)..(13): phosphocoumaryl amino propionic acid
RRRRRRRRRXDEXLI

SEQ ID NO: 95 - protein, 15 aa, Artificial Sequence
  Synthetic Construct
  MISC_FEATURE (10)..(10): 8-amino-3,6-dioxaoctanoic acid
  MISC_FEATURE (13)..(13): phosphocoumaryl amino propionic acid
RKKRRQRRRXDEXLI

SEQ ID NO: 96 - protein, 22 aa, Artificial Sequence
  Synthetic Construct
  MISC_FEATURE (17)..(17): 8-amino-3,6-dioxaoctanoic acid
  MISC_FEATURE (20)..(20): phosphocoumaryl amino propionic acid
RQIKIWFQNRRMKWKKXDEXLI

SEQ ID NO: 97 - protein, 16 aa, Artificial Sequence
  Synthetic Construct
  MISC_FEATURE (1)..(1): trimesic acid
  MISC_FEATURE (12)..(12): L-2-naphthylalanine
  MISC_FEATURE (14)..(14): L-2,3-diaminopropionic acid
  MISC_FEATURE (16)..(16): rhodamine B
XAAAAAKRRRRXFXKX

SEQ ID NO: 98 - protein, 18 aa, Artificial Sequence
  Synthetic Construct
  MISC_FEATURE (1)..(1): trimesic acid
  MISC_FEATURE (14)..(14): L-2-naphthylalanine
  MISC_FEATURE (16)..(16): L-2,3-diaminopropionic acid
  MISC_FEATURE (18)..(18): rhodamine B
XAAAAAAAKRRRRXFXKX

SEQ ID NO: 99 - protein, 15 aa, Artificial Sequence
  Synthetic Construct
  MISC_FEATURE (1)..(1): trimesic acid
  misc_feature (11)..(11): Xaa can be any naturally occurring amino acid
  MISC_FEATURE (12)..(12): L-2-naphthylalanine
  misc_feature (13)..(13): Xaa can be any naturally occurring amino acid
  MISC_FEATURE (14)..(14): L-2,3-diaminopropionic acid
  misc_feature (15)..(15): Xaa can be any naturally occurring amino acid
  MISC_FEATURE (16)..(16): rhodamine B
XRARARRRRRXFXKX

SEQ ID NO: 100 - protein, 16 aa, Artificial Sequence
  Synthetic Construct
  MISC_FEATURE (1)..(1): trimesic acid
  MISC_FEATURE (12)..(12): L-2-naphthylalanine
  MISC_FEATURE (14)..(14): L-2,3-diaminopropionic acid
  MISC_FEATURE (16)..(16): rhodamine B
XDADADKRRRRXFXKX

SEQ ID NO: 101 - protein, 13 aa, Artificial Sequence
  Synthetic Construct
  MISC_FEATURE (10)..(10): L-2-naphthylalanine
  MISC_FEATURE (13)..(13): rhodamine B
AAAAARRRRXFKX

SEQ ID NO: 102 - protein, 15 aa, Artificial Sequence
  Synthetic Construct
  MISC_FEATURE (12)..(12): L-2-naphthylalanine
  MISC_FEATURE (15)..(15): rhodamine B
AAAAAAARRRRXFKX

SEQ ID NO: 103 - protein, 8 aa, Artificial Sequence
  Synthetic Construct
  MISC_FEATURE (2)..(2): L-homoproline
FXRRRRCK

SEQ ID NO: 104 - protein, 8 aa, Artificial Sequence
  Synthetic Construct
  MISC_FEATURE (2)..(2): L-homoproline
  MISC_FEATURE (7)..(7): selenocysteine
FXRRRRXK

SEQ ID NO: 105 - protein, 4 aa, Artificial Sequence
  Synthetic Construct
  MISC_FEATURE (2)..(2): L-norleucine
  MISC_FEATURE (3)..(3): selenocysteine
  MISC_FEATURE (5)..(5): 7-amino-4-methylcourmarin
DXXD

SEQ ID NO: 106 - protein, 10 aa, Artificial Sequence
  Synthetic Construct
  MISC_FEATURE (5)..(5): L-homoproline
  MISC_FEATURE (8)..(8): L-norleucine
RRRRXFDXCD

SEQ ID NO: 107 - protein, 10 aa, Artificial Sequence
  Synthetic Construct
  MISC_FEATURE (5)..(5): L-homoproline
  MISC_FEATURE (8)..(8): L-norleucine
RRRRXFDXCD

SEQ ID NO: 108 - protein, 10 aa, Artificial Sequence
  Synthetic Construct
  MISC_FEATURE (5)..(5): L-homoproline
  MISC_FEATURE (8)..(8): L-norleucine
  MISC_FEATURE (9)..(9): selenocysteine
RRRRXFDXXD

SEQ ID NO: 109 - protein, 14 aa, Artificial Sequence
  Synthetic Construct
  MISC_FEATURE (11)..(11): L-norleucine
  MISC_FEATURE (12)..(12): selenocysteine
  MISC_FEATURE (14)..(14): 7-amino-4-methylcourmarin
RRRRRRRRRDXXCX

SEQ ID NO: 110 - protein, 12 aa, Artificial Sequence
  Synthetic Construct
CRRRRFWQCTRV

SEQ ID NO: 111 - protein, 12 aa, Artificial Sequence
  Synthetic Construct
  MISC_FEATURE (1)..(1): selenocysteine
  MISC_FEATURE (9)..(9): selenocysteine
XRRRRFWQXTRV

SEQ ID NO: 112 - protein, 9 aa, Artificial Sequence
  Synthetic Construct
CRRRRFWQC

SEQ ID NO: 113 - protein, 9 aa, Artificial Sequence
  Synthetic Construct
  MISC_FEATURE (2)..(2): L-2-naphthylalanine
FXRRRRPTP

SEQ ID NO: 114 - protein, 9 aa, Artificial Sequence
  Synthetic Construct
  MISC_FEATURE (2)..(2): L-2-naphthylalanine
FXRRRRPCP

SEQ ID NO: 115 - protein, 12 aa, Artificial Sequence
  Synthetic Construct
  MISC_FEATURE (4)..(4): L-4-(phosphonodifluoromethyl)phenylalanine
  MISC_FEATURE (10)..(10): L-beta-naphthylalanine
TNVXARRRRXFQ

SEQ ID NO: 116 - protein, 12 aa, Artificial Sequence
  Synthetic Construct
  MISC_FEATURE (4)..(4): L-4-(phosphonodifluoromethyl)phenylalanine
  MISC_FEATURE (10)..(10): L-beta-naphthylalanine
SVPXHRRRRXFQ

SEQ ID NO: 117 - protein, 12 aa, Artificial Sequence
  Synthetic Construct
  MISC_FEATURE (3)..(3): L-phenylglycine
  MISC_FEATURE (4)..(4): L-4-(phosphonodifluoromethyl)phenylalanine
  MISC_FEATURE (5)..(5): L-norleucine
  MISC_FEATURE (10)..(10): L-beta-naphthylalanine
IPXXXRRRRXFQ

SEQ ID NO: 118 - protein, 8 aa, Artificial Sequence
  Synthetic Construct
  MISC_FEATURE (2)..(2): sarcosine
  MISC_FEATURE (3)..(3): D-phosphothreonine
  MISC_FEATURE (4)..(4): L-pipecolic acid
  MISC_FEATURE (5)..(5): L-beta-naphthylalanine
AXXXXYQK

SEQ ID NO: 119 - protein, 17 aa, Artificial Sequence
  Synthetic Construct
  MISC_FEATURE (1)..(1): trimesic acid
  MISC_FEATURE (3)..(3): sarcosine
  MISC_FEATURE (4)..(4): D-phosphothreonine
  MISC_FEATURE (5)..(5): L-pipecolic acid
  MISC_FEATURE (6)..(6): L-beta-naphthylalanine
  MISC_FEATURE (9)..(9): L-2,3-diaminopropionic acid
  misc_feature (11)..(11): Xaa can be any naturally occurring amino acid
  MISC_FEATURE (16)..(16): L-2,3-diaminopropionic acid
XAXXXXRAXFXRRRRXK

SEQ ID NO: 120 - protein, 19 aa, Artificial Sequence
  Synthetic Construct
  MISC_FEATURE (1)..(1): trimesic acid
  MISC_FEATURE (3)..(3): sarcosine
  MISC_FEATURE (4)..(4): D-phosphothreonine
  MISC_FEATURE (5)..(5): L-pipecolic acid
  MISC_FEATURE (6)..(6): L-beta-naphthylalanine
  MISC_FEATURE (10)..(10): L-2,3-diaminopropionic acid
  MISC_FEATURE (13)..(13): L-beta-naphthylalanine
  MISC_FEATURE (18)..(18): L-2,3-diaminopropionic acid
XAXXXXRAAXFNXRRRRXK

SEQ ID NO: 121 - protein, 18 aa, Artificial Sequence
  Synthetic Construct
  MISC_FEATURE (1)..(1): trimesic acid
  MISC_FEATURE (3)..(3): sarcosine
  MISC_FEATURE (5)..(5): L-pipecolic acid
  MISC_FEATURE (6)..(6): L-beta-naphthylalanine
  MISC_FEATURE (10)..(10): L-2,3-diaminopropionic acid
  MISC_FEATURE (12)..(12): L-beta-naphthylalanine
  MISC_FEATURE (17)..(17): L-2,3-diaminopropionic acid
XAXTXXRAAXFXRRRRXK

SEQ ID NO: 122 - protein, 18 aa, Artificial Sequence
  Synthetic Construct
  MISC_FEATURE (1)..(1): trimesic acid
  MISC_FEATURE (3)..(3): sarcosine
  MISC_FEATURE (6)..(6): L-beta-naphthylalanine
  MISC_FEATURE (10)..(10): L-2,3-diaminopropionic acid
  misc_feature (12)..(12): Xaa can be any naturally occurring amino acid
  MISC_FEATURE (17)..(17): L-2,3-diaminopropionic acid
XAXTAXRAAXFXRRRRXK

SEQ ID NO: 123 - protein, 8 aa, Artificial Sequence
  Synthetic Construct
  MISC_FEATURE (2)..(2): L-homoproline
FXRRRRCK

SEQ ID NO: 124 - protein, 16 aa, Artificial Sequence
  Synthetic Construct
RQIKIWFQNRRMKWKK

SEQ ID NO: 125 - protein, 5 aa, Artificial Sequence
  Synthetic Construct
  MISC_FEATURE (3)..(3): 2-aminobutyric acid
  MISC_FEATURE (5)..(5): 7-amino-4-methylcourmarin
DMXDX

SEQ ID NO: 126 - protein, 10 aa, Artificial Sequence
  Synthetic Construct
  MISC_FEATURE (5)..(5): L-homoproline
  MISC_FEATURE (8)..(8): L-norleucine
RRRRXFDXCD

SEQ ID NO: 127 - protein, 10 aa, Artificial Sequence
  Synthetic Construct
  MISC_FEATURE (5)..(5): L-homoproline
  MISC_FEATURE (8)..(8): L-norleucine
RRRRXFDXCD

SEQ ID NO: 128 - protein, 10 aa, Artificial Sequence
  Synthetic Construct
  MISC_FEATURE (5)..(5): L-homoproline
  MISC_FEATURE (8)..(8): L-norleucine
  MISC_FEATURE (9)..(9): selenocysteine
RRRRXFDXXD

SEQ ID NO: 129 - protein, 14 aa, Artificial Sequence
  Synthetic Construct
  MOD_RES (11)..(11): Nle
  MISC_FEATURE (12)..(12): 2-aminobutyric acid
  MISC_FEATURE (14)..(14): 7-amino-4-methylcourmarin
RRRRRRRRRDXXDX

SEQ ID NO: 130 - protein, 12 aa, Artificial Sequence
  Synthetic Construct
CRRRRFWQCTRV

SEQ ID NO: 131 - protein, 12 aa, Artificial Sequence
  Synthetic Construct
  MISC_FEATURE (1)..(1): 2-aminobutyric acid
  MISC_FEATURE (9)..(9): 2-aminobutyric acid
XRRRRFWQXTRV

SEQ ID NO: 132 - protein, 12 aa, Artificial Sequence
  Synthetic Construct
CRRRRFWQCTRV

SEQ ID NO: 133 - protein, 9 aa, Artificial Sequence
  Synthetic Construct
RRRRRRRRR

SEQ ID NO: 134 - protein, 11 aa, Artificial Sequence
  Synthetic Construct
YGRKKRRQRRR

SEQ ID NO: 135 - protein, 16 aa, Artificial Sequence
  Synthetic Construct
RQIKIWFQNRRMKWKK

SEQ ID NO: 136 - protein, 6 aa, Artificial Sequence
  Synthetic Construct
  MISC_FEATURE (2)..(2): L-homoproline
  MISC_FEATURE (4)..(4): L-4-(phosphonodifluoromethyl)phenylalanine
PXGXYR

SEQ ID NO: 137 - protein, 6 aa, Artificial Sequence
  Synthetic Construct
  MISC_FEATURE (2)..(2): L-homoproline
  MISC_FEATURE (4)..(4): L-4-(phosphonodifluoromethyl)phenylalanine
  MISC_FEATURE (5)..(5): L-4-(phosphonodifluoromethyl)phenylalanine
SXIXXR

SEQ ID NO: 138 - protein, 6 aa, Artificial Sequence
  Synthetic Construct
  MISC_FEATURE (4)..(4): L-4-(phosphonodifluoromethyl)phenylalanine
IHIXIR

SEQ ID NO: 139 - protein, 6 aa, Artificial Sequence
  Synthetic Construct
  MISC_FEATURE (4)..(4): L-4-(phosphonodifluoromethyl)phenylalanine
  MISC_FEATURE (5)..(5): L-homoproline
AAIXXR

SEQ ID NO: 140 - protein, 6 aa, Artificial Sequence
  Synthetic Construct
  MISC_FEATURE (1)..(1): L-4-fluorophenylalanine
  MISC_FEATURE (3)..(3): L-homoproline
  MISC_FEATURE (4)..(4): L-4-(phosphonodifluoromethyl)phenylalanine
XSXXVR

SEQ ID NO: 141 - protein, 6 aa, Artificial Sequence
  Synthetic Construct
  MISC_FEATURE (1)..(1): L-homoproline
  MISC_FEATURE (4)..(4): L-4-(phosphonodifluoromethyl)phenylalanine
XNPXAR

SEQ ID NO: 142 - protein, 6 aa, Artificial Sequence
  Synthetic Construct
  MISC_FEATURE (2)..(2): L-phenylglycine
  MISC_FEATURE (4)..(4): L-4-(phosphonodifluoromethyl)phenylalanine
YXAXGR

SEQ ID NO: 143 - protein, 6 aa, Artificial Sequence
  Synthetic Construct
  MISC_FEATURE (4)..(4): L-4-(phosphonodifluoromethyl)phenylalanine
AHIXAR

SEQ ID NO: 144 - protein, 6 aa, Artificial Sequence
  Synthetic Construct
  MISC_FEATURE (4)..(4): L-4-(phosphonodifluoromethyl)phenylalanine
GNGXPR

SEQ ID NO: 145 - protein, 6 aa, Artificial Sequence
  Synthetic Construct
  MISC_FEATURE (3)..(3): L-homoproline
  MISC_FEATURE (4)..(4): L-4-(phosphonodifluoromethyl)phenylalanine
FQXXIR

SEQ ID NO: 146 - protein, 6 aa, Artificial Sequence
  Synthetic Construct
  MISC_FEATURE (4)..(4): L-4-(phosphonodifluoromethyl)phenylalanine
SPGXHR

SEQ ID NO: 147 - protein, 6 aa, Artificial Sequence
  Synthetic Construct
  MISC_FEATURE (1)..(1): L-homoproline
  MISC_FEATURE (4)..(4): L-4-(phosphonodifluoromethyl)phenylalanine
XYIXHR

SEQ ID NO: 148 - protein, 6 aa, Artificial Sequence
  Synthetic Construct
  MISC_FEATURE (4)..(4): L-4-(phosphonodifluoromethyl)phenylalanine
SVPXHR

SEQ ID NO: 149 - protein, 6 aa, Artificial Sequence
  Synthetic Construct
  MISC_FEATURE (4)..(4): L-4-(phosphonodifluoromethyl)phenylalanine
AIPXNR

SEQ ID NO: 150 - protein, 6 aa, Artificial Sequence
  Synthetic Construct
  MISC_FEATURE (1)..(1): L-4-fluorophenylalanine
  MISC_FEATURE (4)..(4): L-4-(phosphonodifluoromethyl)phenylalanine
XSIXQF

SEQ ID NO: 151 - protein, 6 aa, Artificial Sequence
  Synthetic Construct
  MISC_FEATURE (3)..(3): L-phenylglycine
  MISC_FEATURE (4)..(4): L-4-(phosphonodifluoromethyl)phenylalanine
AAXXFR

SEQ ID NO: 152 - protein, 6 aa, Artificial Sequence
  Synthetic Construct
  MISC_FEATURE (3)..(3): L-phenylglycine
  MISC_FEATURE (4)..(4): L-4-(phosphonodifluoromethyl)phenylalanine
  MISC_FEATURE (5)..(5): L-phenylglycine
NTXXXR

SEQ ID NO: 153 - protein, 6 aa, Artificial Sequence
  Synthetic Construct
  MISC_FEATURE (3)..(3): L-phenylglycine
  MISC_FEATURE (4)..(4): L-4-(phosphonodifluoromethyl)phenylalanine
  MISC_FEATURE (5)..(5): L-norleucine
IPXXXR

SEQ ID NO: 154 - protein, 6 aa, Artificial Sequence
  Synthetic Construct
  MISC_FEATURE (2)..(2): L-homoproline
  MISC_FEATURE (3)..(3): L-4-fluorophenylalanine
  MISC_FEATURE (4)..(4): L-4-(phosphonodifluoromethyl)phenylalanine
  MISC_FEATURE (5)..(5): L-homoproline
QXXXXR

SEQ ID NO: 155 - protein, 6 aa, Artificial Sequence
  Synthetic Construct
  MISC_FEATURE (3)..(3): L-4-fluorophenylalanine
  MISC_FEATURE (4)..(4): L-4-(phosphonodifluoromethyl)phenylalanine
NAXXGR

SEQ ID NO: 156 - protein, 6 aa, Artificial Sequence
  Synthetic Construct
  MISC_FEATURE (4)..(4): L-4-(phosphonodifluoromethyl)phenylalanine
NTYXAR

SEQ ID NO: 157 - protein, 6 aa, Artificial Sequence
  Synthetic Construct
  MISC_FEATURE (3)..(3): L-phenylglycine
  MISC_FEATURE (4)..(4): L-4-(phosphonodifluoromethyl)phenylalanine
EAXXVR

SEQ ID NO: 158 - protein, 6 aa, Artificial Sequence
  Synthetic Construct
  MISC_FEATURE (3)..(3): L-phenylglycine
  MISC_FEATURE (4)..(4): L-4-(phosphonodifluoromethyl)phenylalanine
IVXXAR

SEQ ID NO: 159 - protein, 6 aa, Artificial Sequence
  Synthetic Construct
  MISC_FEATURE (3)..(3): L-phenylglycine
  MISC_FEATURE (4)..(4): L-4-(phosphonodifluoromethyl)phenylalanine
YTXXAR

SEQ ID NO: 160 - protein, 6 aa, Artificial Sequence
  Synthetic Construct
  MISC_FEATURE (2)..(2): L-homoproline
  MISC_FEATURE (3)..(3): L-phenylglycine
  MISC_FEATURE (4)..(4): L-4-(phosphonodifluoromethyl)phenylalanine
NXXXIR

SEQ ID NO: 161 - protein, 6 aa, Artificial Sequence
  Synthetic Construct
  MISC_FEATURE (1)..(1): L-homoproline
  MISC_FEATURE (4)..(4): L-4-(phosphonodifluoromethyl)phenylalanine
XNWXHR

SEQ ID NO: 162 - protein, 6 aa, Artificial Sequence
  Synthetic Construct
  MISC_FEATURE (2)..(2): L-homoproline
  MISC_FEATURE (4)..(4): L-4-(phosphonodifluoromethyl)phenylalanine
YXVXIR

SEQ ID NO: 163 - protein, 6 aa, Artificial Sequence
  Synthetic Construct
  MISC_FEATURE (4)..(4): L-4-(phosphonodifluoromethyl)phenylalanine
NSAXGR

SEQ ID NO: 164 - protein, 6 aa, Artificial Sequence
  Synthetic Construct
  MISC_FEATURE (4)..(4): L-4-(phosphonodifluoromethyl)phenylalanine
TNVXAR

SEQ ID NO: 165 - protein, 6 aa, Artificial Sequence
  Synthetic Construct
  MISC_FEATURE (4)..(4): L-4-(phosphonodifluoromethyl)phenylalanine
NTVXTR

SEQ ID NO: 166 - protein, 6 aa, Artificial Sequence
  Synthetic Construct
  MISC_FEATURE (4)..(4): L-4-(phosphonodifluoromethyl)phenylalanine
SITXYR

SEQ ID NO: 167 - protein, 6 aa, Artificial Sequence
  Synthetic Construct
  MISC_FEATURE (2)..(2): L-4-fluorophenylalanine
  MISC_FEATURE (4)..(4): L-4-(phosphonodifluoromethyl)phenylalanine
NXNXLR

SEQ ID NO: 168 - protein, 6 aa, Artificial Sequence
  Synthetic Construct
  MISC_FEATURE (4)..(4): L-4-(phosphonodifluoromethyl)phenylalanine
  MISC_FEATURE (5)..(5): L-norleucine
YNNXXR

SEQ ID NO: 169 - protein, 6 aa, Artificial Sequence
  Synthetic Construct
  MISC_FEATURE (4)..(4): L-4-(phosphonodifluoromethyl)phenylalanine
NYNXGR

SEQ ID NO: 170 - protein, 6 aa, Artificial Sequence
  Synthetic Construct
  MISC_FEATURE (4)..(4): L-4-(phosphonodifluoromethyl)phenylalanine
AWNXAR

SEQ ID NO: 171 - protein, 6 aa, Artificial Sequence
  Synthetic Construct
  MISC_FEATURE (4)..(4): L-4-(phosphonodifluoromethyl)phenylalanine
VTHXYR

SEQ ID NO: 172 - protein, 6 aa, Artificial Sequence
  Synthetic Construct
  MISC_FEATURE (2)..(2): L-phenylglycine
  MISC_FEATURE (4)..(4): L-4-(phosphonodifluoromethyl)phenylalanine
  MISC_FEATURE (5)..(5): L-homoproline
PXHXXR

SEQ ID NO: 173 - protein, 6 aa, Artificial Sequence
  Synthetic Construct
  MISC_FEATURE (2)..(2): L-phenylglycine
  MISC_FEATURE (4)..(4): L-4-(phosphonodifluoromethyl)phenylalanine
NXHXGR

SEQ ID NO: 174 - protein, 6 aa, Artificial Sequence
  Synthetic Construct
  MISC_FEATURE (4)..(4): L-4-(phosphonodifluoromethyl)phenylalanine
PAHXGR

SEQ ID NO: 175 - protein, 6 aa, Artificial Sequence
  Synthetic Construct
  MISC_FEATURE (4)..(4): L-4-(phosphonodifluoromethyl)phenylalanine
AYHXIR

SEQ ID NO: 176 - protein, 6 aa, Artificial Sequence
  Synthetic Construct
  MISC_FEATURE (2)..(2): L-homoproline
  MISC_FEATURE (4)..(4): L-4-(phosphonodifluoromethyl)phenylalanine
NXEXYR

SEQ ID NO: 177 - protein, 6 aa, Artificial Sequence
  Synthetic Construct
  MISC_FEATURE (4)..(4): L-4-(phosphonodifluoromethyl)phenylalanine
VSSXTR

SEQ ID NO: 178 - protein, 12 aa, Artificial Sequence
  Synthetic Construct
  MISC_FEATURE (4)..(4): L-4-(phosphonodifluoromethyl)phenylalanine
  MISC_FEATURE (10)..(10): L-beta-naphthylalanine
TNVXARRRRXFQ

SEQ ID NO: 179 - protein, 12 aa, Artificial Sequence
  Synthetic Construct
  MISC_FEATURE (4)..(4): L-4-(phosphonodifluoromethyl)phenylalanine
  MISC_FEATURE (10)..(10): L-beta-naphthylalanine
SVPXHRRRRXFQ

SEQ ID NO: 180 - protein, 12 aa, Artificial Sequence
  Synthetic Construct
  MISC_FEATURE (3)..(3): L-phenylglycine
  MISC_FEATURE (4)..(4): L-4-(phosphonodifluoromethyl)phenylalanine
  MISC_FEATURE (5)..(5): L-norleucine
  MISC_FEATURE (10)..(10): L-beta-naphthylalanine
IPXXXRRRRXFQ

SEQ ID NO: 181 - protein, 8 aa, Artificial Sequence
  Synthetic Construct
  MISC_FEATURE (2)..(2): sarcosine
  MISC_FEATURE (3)..(3): D-phosphothreonine
  MISC_FEATURE (4)..(4): L-homoproline
  MISC_FEATURE (5)..(5): L-beta-naphthylalanine
AXXXXYQK

SEQ ID NO: 182 - protein, 16 aa, Artificial Sequence
  Synthetic Construct
  MISC_FEATURE (1)..(1): trimesic acid
  MISC_FEATURE (3)..(3): sarcosine
  MISC_FEATURE (4)..(4): D-phosphothreonine
  MISC_FEATURE (5)..(5): L-homoproline
  MISC_FEATURE (6)..(6): L-beta-naphthylalanine
  MISC_FEATURE (9)..(9): L-2,3-diaminopropionic acid
  MISC_FEATURE (11)..(11): L-beta-naphthylalanine
  MISC_FEATURE (16)..(16): L-2,3-diaminopropionic acid
XAXXXXRAXFXRRRRK

SEQ ID NO: 183 - protein, 18 aa, Artificial Sequence
  Synthetic Construct
  MISC_FEATURE (1)..(1): trimesic acid
  MISC_FEATURE (3)..(3): sarcosine
  MISC_FEATURE (4)..(4): D-phosphothreonine
  MISC_FEATURE (5)..(5): L-homoproline
  MISC_FEATURE (6)..(6): L-beta-naphthylalanine
  MISC_FEATURE (10)..(10): L-2,3-diaminopropionic acid
  MISC_FEATURE (12)..(12): L-beta-naphthylalanine
  MISC_FEATURE (17)..(17): L-2,3-diaminopropionic acid
XAXXXXRAAXFXRRRRXK

SEQ ID NO: 184 - protein, 18 aa, Artificial Sequence
  Synthetic Construct
  MISC_FEATURE (1)..(1): trimesic acid
  MISC_FEATURE (3)..(3): sarcosine
  MISC_FEATURE (5)..(5): L-homoproline
  MISC_FEATURE (6)..(6): L-beta-naphthylalanine
  MISC_FEATURE (10)..(10): L-2,3-diaminopropionic acid
  MISC_FEATURE (12)..(12): L-beta-naphthylalanine
  MISC_FEATURE (17)..(17): L-2,3-diaminopropionic acid
XAXTXXRAAXFXRRRRXK

SEQ ID NO: 185 - protein, 18 aa, Artificial Sequence
  Synthetic Construct
  MISC_FEATURE (1)..(1): trimesic acid
  MISC_FEATURE (3)..(3): sarcosine
  MISC_FEATURE (6)..(6): L-beta-naphthylalanine
  MISC_FEATURE (10)..(10): L-2,3-diaminopropionic acid
  MISC_FEATURE (12)..(12): L-beta-naphthylalanine
  MISC_FEATURE (17)..(17): L-2,3-diaminopropionic acid
XAXTAXRAAXFXRRRRXK

SEQ ID NO: 186 - protein, 7 aa, Artificial Sequence
  Synthetic Construct
  MISC_FEATURE (2)..(2): L-naphthylalanine
FXRRRRQ

SEQ ID NO: 187 - protein, 8 aa, Artificial Sequence
  Synthetic Construct
  MISC_FEATURE (3)..(3): L-naphthylalanine
FFXRRRRQ

SEQ ID NO: 188 - protein, 7 aa, Artificial Sequence
  Synthetic Construct
  MISC_FEATURE (2)..(2): L-naphthylalanine
FXRRRRQ

SEQ ID NO: 189 - protein, 8 aa, Artificial Sequence
  Synthetic Construct
  MISC_FEATURE (2)..(2): L-naphthylalanine
FXRRRRRQ

SEQ ID NO: 190 - protein, 8 aa, Artificial Sequence
  Synthetic Construct
  MISC_FEATURE (2)..(2): D-naphthylalanine
  misc_feature (3)..(3): Xaa can be any naturally occurring amino acid
CFXRRRRQ

SEQ ID NO: 191 - protein, 7 aa, Artificial Sequence
  Synthetic Construct
  MISC_FEATURE (2)..(2): D-naphthylalanine
FXRRRRQ

SEQ ID NO: 192 - protein, 8 aa, Artificial Sequence
  Synthetic Construct
  MISC_FEATURE (2)..(2): L-naphthylalanine
FXRRRRRQ

SEQ ID NO: 193 - protein, 7 aa, Artificial Sequence
  Synthetic Construct
  MISC_FEATURE (5)..(5): L-naphthylalanine
RRFRXRQ

SEQ ID NO: 194 - protein, 8 aa, Artificial Sequence
  Synthetic Construct
  MISC_FEATURE (3)..(3): L-naphthylalanine
FFXRRRRQ

SEQ ID NO: 195 - protein, 8 aa, Artificial Sequence
  Synthetic Construct
  MISC_FEATURE (6)..(6): L-naphthylalanine
RFRFRXRQ

SEQ ID NO: 196 - protein, 6 aa, Artificial Sequence
  Synthetic Construct
  MISC_FEATURE (2)..(2): L-naphthylalanine
FXRRRQ

SEQ ID NO: 197 - protein, 7 aa, Artificial Sequence
  Synthetic Construct
  MISC_FEATURE (6)..(6): L-naphthylalanine
FRRRRXQ

SEQ ID NO: 198 - protein, 7 aa, Artificial Sequence
  Synthetic Construct
  MISC_FEATURE (5)..(5): L-naphthylalanine
RRFRXRQ

SEQ ID NO: 199 - protein, 7 aa, Artificial Sequence
  Synthetic Construct
  MISC_FEATURE (3)..(3): L-naphthylalanine
RRXFRRQ

SEQ ID NO: 200 - protein, 18 aa, Artificial Sequence
  Synthetic Construct
  MISC_FEATURE (1)..(1): trimesic acid
  MISC_FEATURE (3)..(3): sarcosine
  MISC_FEATURE (4)..(4): D-phosphothreonine
  MISC_FEATURE (5)..(5): L-homoproline
  MISC_FEATURE (6)..(6): L-beta-naphthylalanine
  MISC_FEATURE (10)..(10): L-2,3-diaminopropionic acid
  MISC_FEATURE (12)..(12): L-beta-naphthylalanine
  MISC_FEATURE (17)..(17): L-2,3-diaminopropionic acid
XAXXXXRAAXFXRRRRXK

SEQ ID NO: 201 - protein, 18 aa, Artificial Sequence
  Synthetic Construct
  MISC_FEATURE (1)..(1): trimesic acid
  MISC_FEATURE (3)..(3): sarcosine
  MISC_FEATURE (5)..(5): L-homoproline
  MISC_FEATURE (6)..(6): L-beta-naphthylalanine
  MISC_FEATURE (10)..(10): L-2,3-diaminopropionic acid
  MISC_FEATURE (12)..(12): L-beta-naphthylalanine
  MISC_FEATURE (17)..(17): L-2,3-diaminopropionic acid
XAXTXXRAAXFXRRRRXK

SEQ ID NO: 202 - protein, 17 aa, Artificial Sequence
  Synthetic Construct
  MISC_FEATURE (1)..(1): trimesic acid
  MISC_FEATURE (3)..(3): sarcosine
  MISC_FEATURE (5)..(5): L-homoproline
  MISC_FEATURE (6)..(6): L-beta-naphthylalanine
  MISC_FEATURE (10)..(10): L-2,3-diaminopropionic acid
  MISC_FEATURE (12)..(12): L-beta-naphthylalanine
  MISC_FEATURE (17)..(17): L-2,3-diaminopropionic acid
XPXDXXRAAXFXRRRRK

SEQ ID NO: 203 - protein, 18 aa, Artificial Sequence
  Synthetic Construct
  MISC_FEATURE (1)..(1): trimesic acid
  MISC_FEATURE (3)..(3): L-4-fluorophenylalanine
  MISC_FEATURE (5)..(5): L-homoproline
  MISC_FEATURE (6)..(6): L-beta-naphthylalanine
  MISC_FEATURE (10)..(10): L-2,3-diaminopropionic acid
  MISC_FEATURE (12)..(12): L-beta-naphthylalanine
  MISC_FEATURE (17)..(17): L-2,3-diaminopropionic acid
XFXTXXRAAXFXRRRRXK

SEQ ID NO: 204 - protein, 17 aa, Artificial Sequence
  Synthetic Construct
  MISC_FEATURE (1)..(1): trimesic acid
  MISC_FEATURE (2)..(2): L-N(alpha)-methylphenylalanine
  MISC_FEATURE (5)..(5): L-homoproline
  MISC_FEATURE (6)..(6): L-beta-naphthylalanine
  MISC_FEATURE (10)..(10): L-2,3-diaminopropionic acid
  MISC_FEATURE (12)..(12): L-beta-naphthylalanine
  MISC_FEATURE (17)..(17): L-2,3-diaminopropionic acid
XXGTXXRAAXFXRRRRK

SEQ ID NO: 205 - protein, 18 aa, Artificial Sequence
  Synthetic Construct
  MISC_FEATURE (1)..(1): trimesic acid
  MISC_FEATURE (2)..(2): L-phenylglycine
  MISC_FEATURE (5)..(5): L-homoproline
  MISC_FEATURE (6)..(6): L-beta-naphthylalanine
  MISC_FEATURE (10)..(10): L-2,3-diaminopropionic acid
  MISC_FEATURE (12)..(12): L-beta-naphthylalanine
  MISC_FEATURE (17)..(17): L-2,3-diaminopropionic acid
XXHEXXRAAXFXRRRRXK

SEQ ID NO: 206 - protein, 18 aa, Artificial Sequence
  Synthetic Construct
  MISC_FEATURE (1)..(1): trimesic acid
  MISC_FEATURE (2)..(2): L-N(alpha)-methylphenylalanine
  MISC_FEATURE (5)..(5): L-homoproline
  MISC_FEATURE (6)..(6): L-beta-naphthylalanine
  MISC_FEATURE (10)..(10): L-2,3-diaminopropionic acid
  MISC_FEATURE (12)..(12): L-beta-naphthylalanine
  MISC_FEATURE (17)..(17): L-2,3-diaminopropionic acid
XXIEXXRAAXFXRRRRXK

SEQ ID NO: 207 - protein, 18 aa, Artificial Sequence
  Synthetic Construct
  MISC_FEATURE (1)..(1): trimesic acid
  MISC_FEATURE (3)..(3): L-phenylglycine
  MISC_FEATURE (5)..(5): L-homoproline
  MISC_FEATURE (6)..(6): L-beta-naphthylalanine
  MISC_FEATURE (10)..(10): L-2,3-diaminopropionic acid
  MISC_FEATURE (12)..(12): L-beta-naphthylalanine
  MISC_FEATURE (17)..(17): L-2,3-diaminopropionic acid
XHXTXXRAAXFXRRRRXK

SEQ ID NO: 208 - protein, 17 aa, Artificial Sequence
  Synthetic Construct
  MISC_FEATURE (1)..(1): trimesic acid
  misc_feature (3)..(3): Xaa can be any naturally occurring amino acid
  MISC_FEATURE (5)..(5): L-homoproline
  MISC_FEATURE (6)..(6): L-beta-naphthylalanine
  MISC_FEATURE (9)..(9): L-2,3-diaminopropionic acid
  MISC_FEATURE (11)..(11): L-beta-naphthylalanine
  MISC_FEATURE (16)..(16): L-2,3-diaminopropionic acid
XPXDXXRAXFXRRRRXK

SEQ ID NO: 209 - protein, 16 aa, Artificial Sequence
  Synthetic Construct
  MISC_FEATURE (1)..(1): trimesic acid
  MISC_FEATURE (3)..(3): sarcosine
  MISC_FEATURE (5)..(5): L-homoproline
  MISC_FEATURE (6)..(6): L-beta-naphthylalanine
  MISC_FEATURE (8)..(8): L-2,3-diaminopropionic acid
  MISC_FEATURE (10)..(10): L-beta-naphthylalanine
  MISC_FEATURE (15)..(15): L-2,3-diaminopropionic acid
XPXDXXRXFXRRRRXK

SEQ ID NO: 210 - protein, 17 aa, Artificial Sequence
  Synthetic Construct
  MISC_FEATURE (1)..(1): trimesic acid
  MISC_FEATURE (3)..(3): L-4-fluorophenylalanine
  MISC_FEATURE (5)..(5): L-homoproline
  MISC_FEATURE (6)..(6): L-beta-naphthylalanine
  MISC_FEATURE (9)..(9): L-2,3-diaminopropionic acid
  misc_feature (11)..(11): Xaa can be any naturally occurring amino acid
  MISC_FEATURE (16)..(16): L-beta-naphthylalanine
XFXTXXRAXFXRRRRXK

SEQ ID NO: 211 - protein, 16 aa, Artificial Sequence
  Synthetic Construct
  MISC_FEATURE (1)..(1): trimesic acid
  MISC_FEATURE (3)..(3): L-4-fluorophenylalanine
  MISC_FEATURE (5)..(5): L-homoproline
  MISC_FEATURE (6)..(6): L-beta-naphthylalanine
  MISC_FEATURE (8)..(8): L-2,3-diaminopropionic acid
  MISC_FEATURE (10)..(10): L-beta-naphthylalanine
  MISC_FEATURE (15)..(15): L-2,3-diaminopropionic acid
XFXTXXRXFXRRRRXK

SEQ ID NO: 212 - protein, 17 aa, Artificial Sequence
  Synthetic Construct
  MISC_FEATURE (1)..(1): trimesic acid
  MISC_FEATURE (3)..(3): sarcosine
  MISC_FEATURE (5)..(5): L-homoproline
  MISC_FEATURE (6)..(6): L-beta-naphthylalanine
  misc_feature (9)..(9): Xaa can be any naturally occurring amino acid
  MISC_FEATURE (10)..(10): L-2,3-diaminopropionic acid
  MISC_FEATURE (11)..(11): L-beta-naphthylalanine
  MISC_FEATURE (16)..(16): L-2,3-diaminopropionic acid
XPXDXXAAXFXRRRRXK

SEQ ID NO: 213 - protein, 18 aa, Artificial Sequence
  Synthetic Construct
  MISC_FEATURE (1)..(1): trimesic acid
  MISC_FEATURE (3)..(3): sarcosine
  MISC_FEATURE (5)..(5): L-homoproline
  MISC_FEATURE (6)..(6): L-beta-naphthylalanine
  MISC_FEATURE (10)..(10): L-2,3-diaminopropionic acid
  MISC_FEATURE (12)..(12): L-beta-naphthylalanine
  MISC_FEATURE (17)..(17): L-2,3-diaminopropionic acid
XPXDXXRAAXFXRRRRXK

SEQ ID NO: 214 - protein, 18 aa, Artificial Sequence
  Synthetic Construct
  MISC_FEATURE (1)..(1): trimesic acid
  MISC_FEATURE (3)..(3): sarcosine
  MISC_FEATURE (5)..(5): L-homoproline
  MISC_FEATURE (6)..(6): L-beta-naphthylalanine
  MISC_FEATURE (10)..(10): L-2,3-diaminopropionic acid
  MISC_FEATURE (12)..(12): L-beta-naphthylalanine
  MISC_FEATURE (17)..(17): L-2,3-diaminopropionic acid
XPXDXXRAAXFXRRRRXK

SEQ ID NO: 215 - protein, 19 aa, Artificial Sequence
  Synthetic Construct
  MISC_FEATURE (1)..(1): trimesic acid
  MISC_FEATURE (3)..(3): sarcosine
  MISC_FEATURE (5)..(5): L-homoproline
  MISC_FEATURE (6)..(6): L-beta-naphthylalanine
  MISC_FEATURE (11)..(11): L-2,3-diaminopropionic acid
  MISC_FEATURE (13)..(13): L-beta-naphthylalanine
  MISC_FEATURE (18)..(18): L-2,3-diaminopropionic acid
XPXDXXRAAAXFXRRRRXK

SEQ ID NO: 216 - protein, 18 aa, Artificial Sequence
  Synthetic Construct
  MISC_FEATURE (1)..(1): trimesic acid
  MISC_FEATURE (3)..(3): sarcosine
  MISC_FEATURE (5)..(5): L-homoproline
  MISC_FEATURE (6)..(6): L-beta-naphthylalanine
  MISC_FEATURE (10)..(10): L-2,3-diaminopropionic acid
  MISC_FEATURE (12)..(12): L-beta-naphthylalanine
  MISC_FEATURE (17)..(17): L-2,3-diaminopropionic acid
XPXDXXRYAXFXRRRRXK

SEQ ID NO: 217 - protein, 18 aa, Artificial Sequence
  Synthetic Construct
  MISC_FEATURE (1)..(1): trimesic acid
  MISC_FEATURE (3)..(3): sarcosine
  MISC_FEATURE (5)..(5): L-homoproline
  MISC_FEATURE (6)..(6): L-beta-naphthylalanine
  MISC_FEATURE (10)..(10): L-2,3-diaminopropionic acid
  MISC_FEATURE (12)..(12): L-beta-naphthylalanine
  MISC_FEATURE (17)..(17): L-2,3-diaminopropionic acid
XPXDXXRVAXFXRRRRXK

SEQ ID NO: 218 - protein, 18 aa, Artificial Sequence
  Synthetic Construct
  MISC_FEATURE (1)..(1): trimesic acid
  MISC_FEATURE (3)..(3): sarcosine
  MISC_FEATURE (5)..(5): L-homoproline
  MISC_FEATURE (6)..(6): L-beta-naphthylalanine
  MISC_FEATURE (10)..(10): L-2,3-diaminopropionic acid
  MISC_FEATURE (12)..(12): L-beta-naphthylalanine
  MISC_FEATURE (17)..(17): L-2,3-diaminopropionic acid
XPXDXXRRAXFXRRRRXK

SEQ ID NO: 219 - protein, 18 aa, Artificial Sequence
  Synthetic Construct
  MISC_FEATURE (1)..(1): trimesic acid
  MISC_FEATURE (3)..(3): sarcosine
  MISC_FEATURE (5)..(5): L-homoproline
  MISC_FEATURE (6)..(6): L-beta-naphthylalanine
  MISC_FEATURE (10)..(10): L-2,3-diaminopropionic acid
  MISC_FEATURE (12)..(12): L-beta-naphthylalanine
  MISC_FEATURE (17)..(17): L-2,3-diaminopropionic acid
XPXDXXRDAXFXRRRRXK

SEQ ID NO: 220 - protein, 18 aa, Artificial Sequence
  Synthetic Construct
  MISC_FEATURE (1)..(1): trimesic acid
  MISC_FEATURE (3)..(3): L-4-fluorophenylalanine
  MISC_FEATURE (5)..(5): L-homoproline
  MISC_FEATURE (6)..(6): L-beta-naphthylalanine
  MISC_FEATURE (10)..(10): L-2,3-diaminopropionic acid
  MISC_FEATURE (12)..(12): L-beta-naphthylalanine
  MISC_FEATURE (17)..(17): L-2,3-diaminopropionic acid
XFXTXXRSFXFXRRRRXK

SEQ ID NO: 221 - protein, 18 aa, Artificial Sequence
  Synthetic Construct
  MISC_FEATURE (1)..(1): trimesic acid
  MISC_FEATURE (3)..(3): sarcosine
  MISC_FEATURE (5)..(5): L-homoproline
  MISC_FEATURE (6)..(6): L-beta-naphthylalanine
  MISC_FEATURE (10)..(10): L-2,3-diaminopropionic acid
  MISC_FEATURE (12)..(12): L-beta-naphthylalanine
  MISC_FEATURE (17)..(17): L-2,3-diaminopropionic acid
XPXDXXRRFXFXRRRRXK

SEQ ID NO: 222 - protein, 18 aa, Artificial Sequence
  Synthetic Construct
  MISC_FEATURE (1)..(1): trimesic acid
  MISC_FEATURE (3)..(3): sarcosine
  MISC_FEATURE (5)..(5): L-homoproline
  MISC_FEATURE (6)..(6): L-beta-naphthylalanine
  MISC_FEATURE (10)..(10): L-2,3-diaminopropionic acid
  MISC_FEATURE (12)..(12): L-beta-naphthylalanine
  MISC_FEATURE (17)..(17): L-2,3-diaminopropionic acid
XPXDXXRRVXFXRRRRXK

SEQ ID NO: 223 - protein, 18 aa, Artificial Sequence
  Synthetic Construct
  MISC_FEATURE (1)..(1): trimesic acid
  MISC_FEATURE (3)..(3): sarcosine
  MISC_FEATURE (5)..(5): L-homoproline
  MISC_FEATURE (6)..(6): L-beta-naphthylalanine
  MISC_FEATURE (10)..(10): L-2,3-diaminopropionic acid
  MISC_FEATURE (12)..(12): L-beta-naphthylalanine
  MISC_FEATURE (17)..(17): L-2,3-diaminopropionic acid
XPXDXXRRRXFXRRRRXK

SEQ ID NO: 224 - protein, 18 aa, Artificial Sequence
  Synthetic Construct
  MISC_FEATURE (1)..(1): trimesic acid
  MISC_FEATURE (3)..(3): sarcosine
  MISC_FEATURE (5)..(5): L-homoproline
  MISC_FEATURE (6)..(6): L-beta-naphthylalanine
  MISC_FEATURE (10)..(10): L-2,3-diaminopropionic acid
  MISC_FEATURE (12)..(12): L-beta-naphthylalanine
  MISC_FEATURE (17)..(17): L-2,3-diaminopropionic acid
XPXDXXRRDXFXRRRRXK

SEQ ID NO: 225 - protein, 18 aa, Artificial Sequence
  Synthetic Construct
  MISC_FEATURE (1)..(1): trimesic acid
  MISC_FEATURE (3)..(3): 4-L-4-fluorophenylalanine
  MISC_FEATURE (5)..(5): L-homoproline
  MISC_FEATURE (6)..(6): L-beta-naphthylalanine
  MISC_FEATURE (10)..(10): L-2,3-diaminopropionic acid
  MISC_FEATURE (12)..(12): L-beta-naphthylalanine
  MISC_FEATURE (17)..(17): L-2,3-diaminopropionic acid
XFXTXXRGAXFXRRRRXK

SEQ ID NO: 226 - protein, 18 aa, Artificial Sequence
  Synthetic Construct
  MISC_FEATURE (1)..(1): trimesic acid
  MISC_FEATURE (3)..(3): 4-L-4-fluorophenylalanine
  MISC_FEATURE (5)..(5): L-homoproline
  MISC_FEATURE (6)..(6): L-beta-naphthylalanine
  MISC_FEATURE (10)..(10): L-2,3-diaminopropionic acid
  MISC_FEATURE (12)..(12): L-beta-naphthylalanine
  MISC_FEATURE (17)..(17): L-2,3-diaminopropionic acid
XFXTXXRAFXFXRRRRXK

SEQ ID NO: 227 - protein, 18 aa, Artificial Sequence
  Synthetic Construct
  MISC_FEATURE (1)..(1): trimesic acid
  MISC_FEATURE (5)..(5): L-homoproline
  MISC_FEATURE (6)..(6): L-beta-naphthylalanine
  MISC_FEATURE (10)..(10): L-2,3-diaminopropionic acid
  MISC_FEATURE (12)..(12): L-beta-naphthylalanine
  MISC_FEATURE (17)..(17): L-2,3-diaminopropionic acid
XFFTXXRAFXFXRRRRXK

SEQ ID NO: 228 - protein, 18 aa, Artificial Sequence
  Synthetic Construct
  MISC_FEATURE (1)..(1): trimesic acid
  MISC_FEATURE (3)..(3): 3,4-difluorophenylalanine
  MISC_FEATURE (5)..(5): L-homoproline
  MISC_FEATURE (6)..(6): L-beta-naphthylalanine
  MISC_FEATURE (10)..(10): L-2,3-diaminopropionic acid
  MISC_FEATURE (12)..(12): L-beta-naphthylalanine
  MISC_FEATURE (17)..(17): L-2,3-diaminopropionic acid
XFXTXXRAFXFXRRRRXK

SEQ ID NO: 229 - protein, 18 aa, Artificial Sequence
  Synthetic Construct
  MISC_FEATURE (1)..(1): trimesic acid
  MISC_FEATURE (3)..(3): 4-chlorophenylalanine
  MISC_FEATURE (5)..(5): L-homoproline
  MISC_FEATURE (6)..(6): L-beta-naphthylalanine
  MISC_FEATURE (10)..(10): L-2,3-diaminopropionic acid
  MISC_FEATURE (12)..(12): L-beta-naphthylalanine
  MISC_FEATURE (17)..(17): L-2,3-diaminopropionic acid
XFXTXXRAFXFXRRRRXK

SEQ ID NO: 230 - protein, 18 aa, Artificial Sequence
  Synthetic Construct
  MISC_FEATURE (1)..(1): trimesic acid
  MISC_FEATURE (5)..(5): L-homoproline
  MISC_FEATURE (6)..(6): L-beta-naphthylalanine
  MISC_FEATURE (10)..(10): L-2,3-diaminopropionic acid
  MISC_FEATURE (12)..(12): L-beta-naphthylalanine
  MISC_FEATURE (17)..(17): L-2,3-diaminopropionic acid
XFHTXXRAFXFXRRRRXK

SEQ ID NO: 231 - protein, 18 aa, Artificial Sequence
  Synthetic Construct
  MISC_FEATURE (1)..(1): trimesic acid
  MISC_FEATURE (3)..(3): 4-bromophenylalanin
  MISC_FEATURE (5)..(5): L-homoproline
  MISC_FEATURE (6)..(6): L-beta-naphthylalanine
  MISC_FEATURE (10)..(10): L-2,3-diaminopropionic acid
  MISC_FEATURE (12)..(12): L-beta-naphthylalanine
  MISC_FEATURE (17)..(17): L-2,3-diaminopropionic acid
XFXTXXRAFXFXRRRRXK

SEQ ID NO: 232 - protein, 18 aa, Artificial Sequence
  Synthetic Construct
  MISC_FEATURE (1)..(1): trimesic acid
  MISC_FEATURE (3)..(3): 4-L-4-fluorophenylalanine
  MISC_FEATURE (5)..(5): L-homoproline
  MISC_FEATURE (6)..(6): L-beta-naphthylalanine
  MISC_FEATURE (10)..(10): L-2,3-diaminopropionic acid
  MISC_FEATURE (12)..(12): L-beta-naphthylalanine
  MISC_FEATURE (17)..(17): L-2,3-diaminopropionic acid
XAXTXXTAAXFXRRRRXK

SEQ ID NO: 233 - protein, 18 aa, Artificial Sequence
  Synthetic Construct
  MISC_FEATURE (1)..(1): trimesic acid
  MISC_FEATURE (3)..(3): 4-L-4-fluorophenylalanine
  MISC_FEATURE (5)..(5): L-homoproline
  MISC_FEATURE (6)..(6): L-beta-naphthylalanine
  MISC_FEATURE (10)..(10): L-2,3-diaminopropionic acid
  MISC_FEATURE (12)..(12): L-beta-naphthylalanine
  MISC_FEATURE (17)..(17): L-2,3-diaminopropionic acid
XVXTXXRAAXFXRRRRXK

SEQ ID NO: 234 - protein, 18 aa, Artificial Sequence
  Synthetic Construct
  MISC_FEATURE (1)..(1): trimesic acid
  MISC_FEATURE (2)..(2): D-2-L-4-fluorophenylalanine
  MISC_FEATURE (3)..(3): L-4-fluorophenylalanine
  MISC_FEATURE (5)..(5): L-homoproline
  MISC_FEATURE (6)..(6): L-beta-naphthylalanine
  MISC_FEATURE (10)..(10): L-2,3-diaminopropionic acid
  MISC_FEATURE (12)..(12): L-beta-naphthylalanine
  MISC_FEATURE (17)..(17): L-2,3-diaminopropionic acid
XXXTXXRAFXFXRRRRXK

SEQ ID NO: 235 - protein, 18 aa, Artificial Sequence
  Synthetic Construct
  MISC_FEATURE (1)..(1): trimesic acid
  MISC_FEATURE (2)..(2): D-3-L-4-fluorophenylalanine
  MISC_FEATURE (3)..(3): L-4-fluorophenylalanine
  MISC_FEATURE (5)..(5): L-homoproline
  MISC_FEATURE (6)..(6): L-beta-naphthylalanine
  MISC_FEATURE (10)..(10): L-2,3-diaminopropionic acid
  MISC_FEATURE (12)..(12): L-beta-naphthylalanine
  MISC_FEATURE (17)..(17): L-2,3-diaminopropionic acid
XXXTXXRAFXFXRRRRXK

SEQ ID NO: 236 - protein, 18 aa, Artificial Sequence
  Synthetic Construct
  MISC_FEATURE (1)..(1): trimesic acid
  MISC_FEATURE (2)..(2): D-4-L-4-fluorophenylalanine
  MISC_FEATURE (3)..(3): L-4-fluorophenylalanine
  MISC_FEATURE (5)..(5): L-homoproline
  MISC_FEATURE (6)..(6): L-beta-naphthylalanine
  MISC_FEATURE (10)..(10): L-2,3-diaminopropionic acid
  MISC_FEATURE (12)..(12): L-beta-naphthylalanine
  MISC_FEATURE (17)..(17): L-2,3-diaminopropionic acid
XXXTXXRAFXFXRRRRXK

SEQ ID NO: 237 - protein, 18 aa, Artificial Sequence
  Synthetic Construct
  MISC_FEATURE (1)..(1): trimesic acid
  MISC_FEATURE (2)..(2): D-4-Cyanophenylalanine
  MISC_FEATURE (3)..(3): L-4-fluorophenylalanine
  MISC_FEATURE (5)..(5): L-homoproline
  MISC_FEATURE (6)..(6): L-beta-naphthylalanine
  MISC_FEATURE (10)..(10): L-2,3-diaminopropionic acid
  MISC_FEATURE (12)..(12): L-beta-naphthylalanine
  MISC_FEATURE (17)..(17): L-2,3-diaminopropionic acid
XXXTXXRAFXFXRRRRXK

SEQ ID NO: 238 - protein, 18 aa, Artificial Sequence
  Synthetic Construct
  MISC_FEATURE (1)..(1): trimesic acid
  MISC_FEATURE (2)..(2): D-4-phenylalanine
  MISC_FEATURE (3)..(3): L-4-fluorophenylalanine
  MISC_FEATURE (5)..(5): L-homoproline
  MISC_FEATURE (6)..(6): L-beta-naphthylalanine
  MISC_FEATURE (10)..(10): L-2,3-diaminopropionic acid
  MISC_FEATURE (12)..(12): L-beta-naphthylalanine
  MISC_FEATURE (17)..(17): L-2,3-diaminopropionic acid
XXXIXXRAFXFXRRRRXK

SEQ ID NO: 239 - protein, 19 aa, Artificial Sequence
  Synthetic Construct
  MISC_FEATURE (1)..(1): trimesic acid
  MISC_FEATURE (2)..(2): D-4-phenylalanine
  MISC_FEATURE (3)..(3): L-4-fluorophenylalanine
  MISC_FEATURE (5)..(5): L-beta-naphthylalanine
  MISC_FEATURE (6)..(6): L-homoproline
  MISC_FEATURE (7)..(7): L-beta-naphthylalanine
  MISC_FEATURE (11)..(11): L-2,3-diaminopropionic acid
  MISC_FEATURE (13)..(13): L-beta-naphthylalanine
  MISC_FEATURE (18)..(18): L-2,3-diaminopropionic acid
XXXDXXXRAFXFXRRRRXK

SEQ ID NO: 240 - protein, 18 aa, Artificial Sequence
  Synthetic Construct
  MISC_FEATURE (1)..(1): trimesic acid
  MISC_FEATURE (2)..(2): D-4-phenylalanine
  MISC_FEATURE (3)..(3): L-4-fluorophenylalanine
  MISC_FEATURE (4)..(4): D-homogluatamine
  MISC_FEATURE (5)..(5): L-homoproline
  MISC_FEATURE (6)..(6): L-beta-naphthylalanine
  MISC_FEATURE (10)..(10): L-2,3-diaminopropionic acid
  MISC_FEATURE (12)..(12): L-beta-naphthylalanine
  MISC_FEATURE (17)..(17): L-2,3-diaminopropionic acid
XXXXXXRAFXFXRRRRXK

SEQ ID NO: 241 - protein, 18 aa, Artificial Sequence
  Synthetic Construct
  MISC_FEATURE (1)..(1): trimesic acid
  MISC_FEATURE (3)..(3): L-4-fluorophenylalanine
  MISC_FEATURE (5)..(5): L-homoproline
  MISC_FEATURE (6)..(6): L-beta-naphthylalanine
  MISC_FEATURE (10)..(10): L-2,3-diaminopropionic acid
  MISC_FEATURE (15)..(15): L-beta-naphthylalanine
  MISC_FEATURE (17)..(17): L-2,3-diaminopropionic acid
XFXTXXRAFXRRRRXFXK

SEQ ID NO: 242 - protein, 18 aa, Artificial Sequence
  Synthetic Construct
  MISC_FEATURE (1)..(1): trimesic acid
  MISC_FEATURE (3)..(3): L-4-fluorophenylalanine
  MISC_FEATURE (5)..(5): L-homoproline
  MISC_FEATURE (6)..(6): L-beta-naphthylalanine
  MISC_FEATURE (10)..(10): L-2,3-diaminopropionic acid
  MISC_FEATURE (13)..(13): L-beta-naphthylalanine
  MISC_FEATURE (17)..(17): L-2,3-diaminopropionic acid
XFXTXXRAFXRRXFRRXK

SEQ ID NO: 243 - protein, 18 aa, Artificial Sequence
  Synthetic Construct
  MISC_FEATURE (1)..(1): trimesic acid
  MISC_FEATURE (3)..(3): L-4-fluorophenylalanine
  MISC_FEATURE (5)..(5): L-homoproline
  MISC_FEATURE (6)..(6): L-beta-naphthylalanine
  MISC_FEATURE (10)..(10): L-2,3-diaminopropionic acid
  MISC_FEATURE (12)..(12): L-beta-naphthylalanine
  MISC_FEATURE (17)..(17): L-2,3-diaminopropionic acid
XFXTXXRAFXRXRFRRXK

SEQ ID NO: 244 - protein, 18 aa, Artificial Sequence
  Synthetic Construct
  MISC_FEATURE (1)..(1): trimesic acid
  MISC_FEATURE (3)..(3): L-4-fluorophenylalanine
  MISC_FEATURE (5)..(5): L-homoproline
  MISC_FEATURE (6)..(6): L-beta-naphthylalanine
  MISC_FEATURE (10)..(10): L-2,3-diaminopropionic acid
  MISC_FEATURE (15)..(15): L-beta-naphthylalanine
  MISC_FEATURE (17)..(17): L-2,3-diaminopropionic acid
XFXTXXRAFXRRRRXFXK

SEQ ID NO: 245 - protein, 8 aa, Artificial Sequence
  Synthetic Construct
  MISC_FEATURE (2)..(2): sarcosine
  MISC_FEATURE (3)..(3): D-phosphothreonine
  MISC_FEATURE (4)..(4): L-homoproline
  MISC_FEATURE (5)..(5): L-beta-naphthylalanine
AXXXXYQK

SEQ ID NO: 246 - protein, 17 aa, Artificial Sequence
  Synthetic Construct
  MISC_FEATURE (1)..(1): trimesic acid
  MISC_FEATURE (3)..(3): sarcosine
  MISC_FEATURE (5)..(5): L-beta-naphthylalanine
  MISC_FEATURE (9)..(9): L-2,3-diaminopropionic acid
  MISC_FEATURE (11)..(11): L-beta-naphthylalanine
  MISC_FEATURE (16)..(16): L-2,3-diaminopropionic acid
XAXAXRAAXFXRRRRXK